European Patent Application EP 4 610 355 A1, published September 3, 2025. Title: GENE EDITING SYSTEM AND USE THEREOF. Applicant: GUANGZHOU REFORGENE MEDICINE CO., LTD. The sequence listing filed with the application follows.

SEQUENCE LISTING (243 sequences)

SEQ ID NO: 1 - protein, 1272 aa, synthetic construct
MYHLSDANHGKHIAGTYYEMAMGNFIHTLSHMLVRAGIKVNKLEDNYSIEREIMNLTAPGAYDAQRAALSRLLYRHFPFFGPIMADHTDHILSSKRKKVQSASDDGNLDLGQELKDEVAGASACQMIRYLATIAGALVYYRNMYSHKNHYDNAQDIAAQQEREQKLALWLDVVFRGARDILLTRKSHPQPDTDFLTQNGTINYYIEKNGKSAYNPNFYFKPGLKTDNGWVMTDFGKFFFCSLFLRRADAERFAAETDLYVGSPFKITAQERARLQEAENKRAADEQARASSAGFPHIVNPRTIGPSESPQNNIIREMLNMHRARIPRERRIDADMSEGILAMDIMNELRRCPLSLYNTLSPEAKASFEKTGVTPEGGIVSNLLVRHSDRYPELALRAIDQMELLPTIRFHVRLGSLRFRFYEKKLIDGSHTLRTVQKAVNGFGRWQEVEPRRVEKYTAIQARCQNDKGIDQFLPDSPTTTPYITDWRTTYNIHANRIGLAWNLPQMSDGIYLPNLDTDKGDNLHRKALIDMPAPMCYLSIFDLPALLFYCHIYTHYHGTKYHLPSAESIIQAKYDALHKFFSFAAAQNHSAEQLREKQLELNLADNEIPDKLRCMMQTKPFFKNGRQQLSPLGYPIMKNWIGVAEQRKHAAQVLRDVANEAADRLASFEKKHQRVVVGGRDNRYGRRGHADIRHGSLARYLATSMVRWQPALDQPGGDKLTSANHRALAGFLSEYGLHGSNINKLRNVLKEAGLIEGSHPHPFLAHVLESAPANIEALYVAYLKHEQSHATALKNKFTDRNGIVQPSEVPAFVRFNSSRWRNDSATTARRYLQTPPAPGSSDSAEHNAPIMLPDGLFTTHIMTLLNKVLGQNDRVPEEDYLRHDLPRIASIINPNGKTYGAAYIIRAWFDQVENQDVQPFYDLPRFYREISLLAPRRKPNQELIRDYFSEEQIAQKIQTVPKKQRSEKVGHTIDTEKDIRRYRLQDITLYLTLLDMLTLMLSRNEAERTDRQMKSSTAERVSNMRLVDFDHSFDFDLLGSTSGEAAYSYLHQRSGITISMPALSLRSYGSIFRVLADSRFETLMDALNRQGVTHVNFGDITSELALYDTLRSHFLLQAHNVEQDAFSAKRGVLENHTSPFFYRSGNLQLDDQGNITNPSTDAIRNHYGELIKILDRYSLKIDKKTKDGKSQDILLRDLMAELRNAAAHNRYPKADFFFRQFDHFLNTCKPTDSNLTAPNYIRTVLEFLKSIVDNNFTPLLHEESPENESKSE

SEQ ID NO: 2 - protein, 1188 aa, synthetic construct
MKEQKKFSLQGVRHVCGSYFNMALNNYCRTLNGVFIKCKIKFALKEDDFPRSLSSLRKIFSSGPIMPQTEKKVAKMIASVDTAMKLKQQLFKHFPMLGPIMDKTISCMNHHKGSSVADAPLDLCMNAILNFGECLYHCRNFYTHFKPYNSPEDLKLQYDIQHIIALNLGTLFDVSRRIGKKREGLTPEELEFLTGKNRFNQVGKKFLERNDWYLKIEKPSDMKDYDKTILSDFGMVYLCSIFLAKNYALRLFDESKLFNKETIRNLFSEEQVRFLKEMLVIYRIRTPRGKQLDSHDSKQALAMDMLNELRKCPRPLYDVLSEEYKKRTFYVPVEHENEKTEEYVKMLRSDDRFPYFTLRYIDDMEKFSRIRFQIRLGSYRFKFYDKMNIDGTPRIRSLQKEINGFGRLSDMENKRKREWKDMFQATEEIDYEDQFGDYQTGVTQFVEDTADTKPYVTNHRAAYNVHSNHIGLIWNDADSIILQDDNKLFFPDLKIDENGKADIYQPSPKASLSVFDFPAMVFYMYLREKTEATKEFPSAEQLIINKYDHLVRFFKDISDGRFGPSENKNAFSKKLKEEYDLKTGEIPEKLLHWLSSESEEDPSEKYAKKLEEEIKLRRERVQRRLEKFNQDLREIRKKDSVPYGKKGHVNIRHSQLAKYLMRSIMEWQPTRNDGKNKLTGQNFNVMTAFLATLGYTSQVKDLRDLFSRANMLEGPNAHPFLKKVLNNNSIKDIQGFYRTYLVEELNQIEDKQRRIAKAKNVKDTVRQFPFAHFNRMRYQKRDEDYYRNLAKRYLNIGDNEKDKAVILLPDGMFTSYIYDLIMKLPENNEKMRINLASDVAHCNSSFLISRFFENIRNDYAQPFYREERTYELFSILNNKKVRNTLQPLFISPHDINIQLTEKEKDGKGRLILQKIDHFCKSITQKGNFNNVEEAKEATSRKLKHLITDCKNNERDIRRYKTQDMVIYLMARDILKDIIPDSEKDKYAKDRKLLLKDVCEEGFLRQAVKMEYEYSIEEKGKRTRTVKITHPNMSLKNYGEFHRLLNDERLKSLLQQLANMDEIDYTDLMGEFADYDQKRSEIFRLAQSIEKHLYEQNEQGLNDEKSDLFYHTRYNGKKIPRRNSFSSLLELIGEEESQMTETDKKQTISIRNAFGHNTYKVSLAEMNATELPNVAKTILKKMEELRNKL

SEQ ID NO: 3 - protein, 893 aa, synthetic construct
MSKDKKTKAKRMGVKALLAHGEDKLTMTTFGKGNRSKIEFTEGYHGRALETPKHFGIRGFEVRRIDENVDLCGDLEEGKTIEALLVNPSEKVGEDYLKLKGTLEKRFFGREFPHDNIRIQLIYNILDIYKILGMNVADILYALGNMQDTELDIDMFGQSLNNEDNLKECLKRMRPYMGYFGDIFKISPKGENIADREHNKKVLRCISVLRNATAHDKQDEYPWFKSSDIYETKIFKADMWKIIKDQYREKIKKVNKDFLSKNAVNMAILFDLLNARDVEQKKQITDEFYRFTIRKDGKNLGMNLVKIREIIIDRYASGLRDKKHDPHRQKINVIADFLIFRALSQNQGIIDKTVSSLRLTKDEEEKDHVYQNAAELVWGMVSNCLTPYFNDPKNKYILKYKDAKTPGDFEDWITSKISEDDGEPFVKVLSFLCNFLEGKEINELLTAYIHKFECIQDFLNVISSLGENVQFQPRFALFNNASFAQNVAVQLRILASIGKMKPDLTEAKRPLYKAAIRMLCPPEKWEKYTSDEWLEKNMLLNSEDRKNDKKKKQVNPFRNFIAGNVIESRRFMYLVRYSKPKAVRAIMQNRSIVNYVLHRLPSEQVHRYASVFPENFADLEQEIDFLTKKLFEFSFEELLHEKDVILNNSRSHKPSLEIERLKAITGLYLSVAYIAIKNIVKANARYYIAFAVFERDKELVKAKDARIQTKIPETDFPDYFCLTQYYLDRDEEKKFPGDPRDKEAFFEHLRKTKRHFSKQWREWLNEKIADAKSSQATGLLLREARNDVEHLNVLRAIPDYIQDFRHGEKGETAMNSYFELYHYLMQRLMLKNTELDLSHWSGWIMRSGRPDRDLIQIAFVSLAYNLPRYRNLTKEHHFDDTVLQKIREKESLD

SEQ ID NO: 4 - DNA, 7930 bp, synthetic construct
  source 1..7930: mol_type = other DNA
cctgcaggcagctgcgcgctcgctcgctcactgaggccgcccgggcgtcgggcgacctttggtcgcccggcctcagtgagcgagcgagcgcgcagagagggagtggccaactccatcactaggggttcctgcggcctctagactcgaggcgttgacattgattattgactagttattaatagtaatcaattacggggtcattagttcatagcccatatatggagttccgcgttacataacttacggtaaatggcccgcctggctgaccgcccaacgacccccgcccattgacgtcaataatgacgtatgttcccatagtaacgccaatagggactttccattgacgtcaatgggtggagtatttacggtaaactgcccacttggcagtacatcaagtgtatcatatgccaagtacgccccctattgacgtcaatgacggtaaatggcccgcctggcattatgcccagtacatgaccttatgggactttcctacttggcagtacatctacgtattagtcatcgctattaccatggtgatgcggttttggcagtacatcaatgggcgtggatagcggtttgactcacggggatttccaagtctccaccccattgacgtcaatgggagtttgttttggcaccaaaatcaacgggactttccaaaatgtcgtaacaactccgccccattgacgcaaatgggcggtaggcgtgtacggtgggaggtctatataagcagagctctctggctaactaccggtgccaccatgccggcagctaagaaaaagaaactggatggcagcgtcgacatgtaccacctgagcgacgccaaccacggcaagcacatcgccggcacctactacgagatggccatgggcaacttcatccacaccctgagccacatgctggtgagagccggcatcaaggtgaacaagctggaggacaactacagcatcgagagagagatcatgaacctgaccgcccccggcgcctacgacgcccagagagccgccctgagcagactgctgtacagacacttccccttcttcggccccatcatggccgaccacaccgaccacatcctgagcagcaagagaaagaaggtgcagagcgccagcgacgacggcaacctggacctgggccaggagctgaaggacgaggtggccggcgccagcgcctgccagatgatcagatacctggccaccatcgccggcgccctggtgtactacagaaacatgtacagccacaagaaccactacgacaacgcccaggacatcgccgcccagcaggagagagagcagaagctggccctgtggctggacgtggtgttcagaggcgccagagacatcctgctgaccagaaagagccacccccagcccgacaccgacttcctgacccagaacggcaccatcaactactacatcgagaagaacggcaagagcgcctacaaccccaacttctacttcaagcccggcctgaaaaccgacaacggctgggtgatgaccgacttcggcaagttcttcttctgcagcctgttcctgagaagagccgacgccgagagattcgccgccgagacagacctgtacgtgggcagccccttcaagatcaccgcccaggagagagccagactgcaggaggccgagaacaagagagccgccgacgagcaggccagagccagcagcgccggcttcccccacatcgtgaaccccagaaccatcggccccagcgagagcccccagaacaacatcatcagagagatgctgaacatgcacagagccagaatccccagagagagaagaatcgacgccgacatgagcgagggcatcctggccatggacatcatgaacgagctgagaagatgccccctgagcctgtacaacaccctgagccccgaggccaaggccagcttcgagaaaaccggcgtgacccccgagggcggcatcgtgagcaacctgctggtgagacacagcgacagataccccgagctggccctgagagccatcgaccagatggagctgctgcccaccatcagattccacgtgagactgggcagcctgagattcagattctacgagaagaagctgatcgacggcagccacaccctgagaaccgtgcagaaggccgtgaacggcttcggcagatggcaggaggtggagcccagaagagtggagaagtacaccgccatccaggccagatgccagaacgacaagggcatcgaccagttcctgcccgacagccccaccaccaccccctacatcaccgactggagaaccacctacaacatccacgccaacagaatcggcctggcctggaacctgccccagatgagcgacggcatctacctgcccaacctggacaccgacaagggcgacaacctgcacagaaaggccctgatcgacatgcccgcccccatgtgctacctgagcatcttcgacctgcccgccctgctgttctactgccacatctacacccactaccacggcaccaagtaccacctgcccagcgccgagagcatcatccaggccaagtacgacgccctgcacaagttcttcagcttcgccgccgcccagaaccacagcgccgagcagctgagagagaagcagctggagctgaacctggccgacaacgagatccccgacaagctgagatgcatgatgcagaccaagcccttcttcaagaacggcagacagcagctgagccccctgggctaccccatcatgaagaactggatcggcgtggccgagcagagaaagcacgccgcccaggtgctgagagacgtggccaacgaggccgccgacagactggccagcttcgagaagaagcaccagagagtggtggtgggcggcagagacaacagatacggcagaagaggccacgccgacatcagacacggcagcctggccagatacctggccaccagcatggtgagatggcagcccgccctggaccagcccggcggcgacaagctgaccagcgccaaccacagagccctggccggcttcctgagcgagtacggcctgcacggcagcaacatcaacaagctgagaaacgtgctgaaggaggccggcctgatcgagggcagccacccccaccccttcctggcccacgtgctggagagcgcccccgccaacatcgaggccctgtacgtggcctacctgaagcacgagcagagccacgccaccgccctgaagaacaagttcaccgacagaaacggcatcgtgcagcccagcgaggtgcccgccttcgtgagattcaacagcagcagatggagaaacgacagcgccaccaccgccagaagatacctgcagaccccccccgcccccggcagcagcgacagcgccgagcacaacgcccccatcatgctgcccgacggcctgttcaccacccacatcatgaccctgctgaacaaggtgctgggccagaacgacagagtgcccgaggaggactacctgagacacgacctgcccagaatcgccagcatcatcaaccccaacggcaagacctacggcgccgcctacatcatcagagcctggttcgaccaggtggagaaccaggacgtgcagcccttctacgacctgcccagattctacagagagatcagcctgctggcccccagaagaaagcccaaccaggagctgatcagagactacttcagcgaggagcagatcgcccagaagatccagaccgtgcccaagaagcagagaagcgagaaggtgggccacaccatcgacaccgagaaggacatcagaagatacagactgcaggacatcaccctgtacctgaccctgctggacatgctgaccctgatgctgagcagaaacgaggccgagagaaccgacagacagatgaagagcagcaccgccgagagagtgagcaacatgagactggtggacttcgaccacagcttcgacttcgacctgctgggcagcaccagcggcgaggccgcctacagctacctgcaccagagaagcggcatcaccatcagcatgcccgccctgagcctgagaagctacggcagcatcttcagagtgctggccgacagcagattcgagacactgatggacgccctgaacagacagggcgtgacccacgtgaacttcggcgacatcaccagcgagctggccctgtacgacaccctgagaagccacttcctgctgcaggcccacaacgtggagcaggacgccttcagcgccaagagaggcgtgctggagaaccacaccagccccttcttctacagaagcggcaacctgcagctggacgaccagggcaacatcaccaaccccagcaccgacgccatcagaaaccactacggcgagctgatcaagatcctggacagatacagcctgaagatcgacaagaaaaccaaggacggcaagagccaggacatcctgctgagagacttgatggccgagctgagaaacgccgccgcccacaacagataccccaaggccgacttcttcttcagacagttcgaccacttcctgaacacctgcaagcccaccgacagcaacctgaccgcccccaactacatcagaaccgtgctggagttcctgaagagcatcgtggacaacaacttcacccccctgctgcacgaggagagccccgagaacgagagcaagagcgagacaggcggcggccccggcggcggcgccgccgccggcagcggcagccctaagaaaaaacgaaaagttggcagcggaagcaaaaggccggcggccacgaaaaaggccggccaggcaaaaaagaaaaagctcgagtacccatacgatgttccagattacgcttgagaattccccttgagcatctgacttctggctaataaaggaaatttattttcattgcaatagtgtgttggaattttttgtgtctctcaggtaccgagggcctatttcccatgattccttcatatttgcatatacgatacaaggctgttagagagataattggaattaatttgactgtaaacacaaagatattagtacaaaatacgtgacgtagaaagtaataatttcttgggtagtttgcagttttaaaattatgttttaaaatggactatcatatgcttaccgtaacttgaaagtatttcgatttcttggctttatatatcttgtggaaaggacgaaacaccggagaccacggcaggtctcagttgtagaagccgttcattcgggacggtatgacaacttttttgcggccgcaggaacccctagtgatggagttggccactccctctctgcgcgctcgctcgctcactgaggccgggcgaccaaaggtcgcccgacgcccgggctttgcccgggcggcctcagtgagcgagcgagcgcgcagctgcctgcaggggcgcctgatgcggtattttctccttacgcatctgtgcggtatttcacaccgcatacgtcaaagcaaccatagtacgcgccctgtagcggcgcattaagcgcggcgggtgtggtggttacgcgcagcgtgaccgctacacttgccagcgccttagcgcccgctcctttcgctttcttcccttcctttctcgccacgttcgccggctttccccgtcaagctctaaatcgggggctccctttagggttccgatttagtgctttacggcacctcgaccccaaaaaacttgatttgggtgatggttcacgtagtgggccatcgccctgatagacggtttttcgccctttgacgttggagtccacgttctttaatagtggactcttgttccaaactggaacaacactcaactctatctcgggctattcttttgatttataagggattttgccgatttcggtctattggttaaaaaatgagctgatttaacaaaaatttaacgcgaattttaacaaaatattaacgtttacaattttatggtgcactctcagtacaatctgctctgatgccgcatagttaagccagccccgacacccgccaacacccgctgacgcgccctgacgggcttgtctgctcccggcatccgcttacagacaagctgtgaccgtctccgggagctgcatgtgtcagaggttttcaccgtcatcaccgaaacgcgcgagacgaaagggcctcgtgatacgcctatttttataggttaatgtcatgataataatggtttcttagacgtcaggtggcacttttcggggaaatgtgcgcggaacccctatttgtttatttttctaaatacattcaaatatgtatccgctcatgagacaataaccctgataaatgcttcaataatattgaaaaaggaagagtatgagtattcaacatttccgtgtcgcccttattcccttttttgcggcattttgccttcctgtttttgctcacccagaaacgctggtgaaagtaaaagatgctgaagatcagttgggtgcacgagtgggttacatcgaactggatctcaacagcggtaagatccttgagagttttcgccccgaagaacgttttccaatgatgagcacttttaaagttctgctatgtggcgcggtattatcccgtattgacgccgggcaagagcaactcggtcgccgcatacactattctcagaatgacttggttgagtactcaccagtcacagaaaagcatcttacggatggcatgacagtaagagaattatgcagtgctgccataaccatgagtgataacactgcggccaacttacttctgacaacgatcggaggaccgaaggagctaaccgcttttttgcacaacatgggggatcatgtaactcgccttgatcgttgggaaccggagctgaatgaagccataccaaacgacgagcgtgacaccacgatgcctgtagcaatggcaacaacgttgcgcaaactattaactggcgaactacttactctagcttcccggcaacaattaatagactggatggaggcggataaagttgcaggaccacttctgcgctcggcccttccggctggctggtttattgctgataaatctggagccggtgagcgtggaagccgcggtatcattgcagcactggggccagatggtaagccctcccgtatcgtagttatctacacgacggggagtcaggcaactatggatgaacgaaatagacagatcgctgagataggtgcctcactgattaagcattggtaactgtcagaccaagtttactcatatatactttagattgatttaaaacttcatttttaatttaaaaggatctaggtgaagatcctttttgataatctcatgaccaaaatcccttaacgtgagttttcgttccactgagcgtcagaccccgtagaaaagatcaaaggatcttcttgagatcctttttttctgcgcgtaatctgctgcttgcaaacaaaaaaaccaccgctaccagcggtggtttgtttgccggatcaagagctaccaactctttttccgaaggtaactggcttcagcagagcgcagataccaaatactgttcttctagtgtagccgtagttaggccaccacttcaagaactctgtagcaccgcctacatacctcgctctgctaatcctgttaccagtggctgctgccagtggcgataagtcgtgtcttaccgggttggactcaagacgatagttaccggataaggcgcagcggtcgggctgaacggggggttcgtgcacacagcccagcttggagcgaacgacctacaccgaactgagatacctacagcgtgagctatgagaaagcgccacgcttcccgaagggagaaaggcggacaggtatccggtaagcggcagggtcggaacaggagagcgcacgagggagcttccagggggaaacgcctggtatctttatagtcctgtcgggtttcgccacctctgacttgagcgtcgatttttgtgatgctcgtcaggggggcggagcctatggaaaaacgccagcaacgcggcctttttacggttcctggccttttgctggccttttgctcacatgt

SEQ ID NO: 5 - DNA, 7679 bp, synthetic construct
  source 1..7679: mol_type = other DNA
cctgcaggcagctgcgcgctcgctcgctcactgaggccgcccgggcgtcgggcgacctttggtcgcccggcctcagtgagcgagcgagcgcgcagagagggagtggccaactccatcactaggggttcctgcggcctctagactcgaggcgttgacattgattattgactagttattaatagtaatcaattacggggtcattagttcatagcccatatatggagttccgcgttacataacttacggtaaatggcccgcctggctgaccgcccaacgacccccgcccattgacgtcaataatgacgtatgttcccatagtaacgccaatagggactttccattgacgtcaatgggtggagtatttacggtaaactgcccacttggcagtacatcaagtgtatcatatgccaagtacgccccctattgacgtcaatgacggtaaatggcccgcctggcattatgcccagtacatgaccttatgggactttcctacttggcagtacatctacgtattagtcatcgctattaccatggtgatgcggttttggcagtacatcaatgggcgtggatagcggtttgactcacggggatttccaagtctccaccccattgacgtcaatgggagtttgttttggcaccaaaatcaacgggactttccaaaatgtcgtaacaactccgccccattgacgcaaatgggcggtaggcgtgtacggtgggaggtctatataagcagagctctctggctaactaccggtgccaccatgccggcagctaagaaaaagaaactggatggcagcgtcgacatgaaggagcagaagaagttcagcctgcagggcgtgagacacgtgtgcggcagctacttcaacatggccctgaacaactactgcagaaccctgaacggcgtgttcatcaagtgcaagatcaagttcgccctgaaggaggacgacttccccagaagcctgagcagcctgagaaagatcttcagcagcggccccatcatgccccagaccgagaagaaggtggccaagatgatcgccagcgtggacaccgccatgaagctgaagcagcagctgttcaagcacttccccatgctgggccccatcatggacaagaccatcagctgcatgaaccaccacaagggcagcagcgtggccgacgcccccctggacctgtgcatgaacgccatcctgaacttcggcgagtgcctgtaccactgcagaaacttctacacccacttcaagccctacaacagccccgaggacctgaagctgcagtacgacatccagcacatcatcgccctgaacctgggcaccctgttcgacgtgagcagaagaatcggcaagaagagagagggcctgacccccgaggagctggagttcctgaccggcaagaacagattcaaccaggtgggcaagaagttcctggagagaaacgactggtacttgaagatcgagaagcccagcgacatgaaggactacgacaagaccatcctgagcgacttcggcatggtgtacctgtgcagcatcttcctggccaagaactacgccctgagactgttcgacgagagcaagctgttcaacaaggagacaatcagaaacctgttcagcgaggagcaggtgagattcctgaaggagatgctggtgatctacagaatcagaacccccagaggcaagcagctggacagccacgacagcaagcaggccctggccatggacatgctgaacgagctgagaaagtgccccagacccctgtacgacgtgctgagcgaggagtacaagaagagaaccttctacgtgcccgtggagcacgagaacgagaaaaccgaggagtacgtgaagatgctgagaagcgacgacagattcccctacttcaccctgagatacatcgacgacatggagaagttcagcagaatcagattccagatcagactgggcagctacagattcaagttctacgacaagatgaacatcgacggcacccccagaatcagaagcctgcagaaggagatcaacggcttcggcagactgagcgacatggagaacaagagaaagagagagtggaaggacatgttccaggccaccgaggagatcgactacgaggaccagttcggcgactaccagaccggcgtgacccagttcgtggaggacaccgccgacaccaagccctacgtgaccaaccacagagccgcctacaacgtgcacagcaaccacatcggcctgatctggaacgacgccgacagcatcatcctgcaggacgacaacaagctgttcttccccgacctgaagatcgacgagaacggcaaggccgacatctaccagcccagccccaaggccagcctgagcgtgttcgacttccccgccatggtgttctacatgtacctgagagagaaaaccgaggccaccaaggagttccccagcgccgagcagctgatcatcaacaagtacgaccacctggtgagattcttcaaggacatcagcgacggcagattcggccccagcgagaacaagaacgccttcagcaagaagctgaaggaggagtacgacctgaaaaccggcgagatccccgagaagctgctgcactggctgagcagcgagagcgaggaggaccccagcgagaagtacgccaagaagctggaggaggagatcaagctgagaagagagagagtgcagagaagattggagaagttcaaccaggacctgagagagatcagaaagaaggacagcgtgccctacggcaagaagggccacgtgaacatcagacacagccagctggccaagtacctgatgagaagcatcatggagtggcagcccaccagaaacgacggcaagaacaagctgaccggccagaacttcaacgtgatgaccgccttcctggccaccctgggctacaccagccaggtgaaggacctgagagacttgttcagcagagccaacatgctggagggccccaacgcccaccccttcctgaagaaggtgctgaacaacaacagcatcaaggacatccagggcttctacagaacctacctggtggaggagctgaaccagatcgaggacaagcagagaagaatcgccaaggccaagaacgtgaaggacaccgtgagacagttccccttcgcccacttcaacagaatgagataccagaagagagacgaggactactacagaaacctggccaagagatacctgaacatcggcgacaacgagaaggacaaggccgtgatcctgctgcccgacggcatgttcaccagctacatctacgacctgatcatgaagctgcccgagaacaacgagaagatgagaatcaacctggccagcgacgtggcccactgcaacagcagcttcctgatcagcagattcttcgagaacatcagaaacgactacgcccagcccttctacagagaggagagaacctacgagctgttcagcatcctgaacaacaagaaggtgagaaacaccctgcagcccctgttcatcagcccccacgacatcaacatccagctgaccgagaaggagaaggacggcaagggcagactgatcctgcagaagatcgaccacttctgcaagagcatcacccagaagggcaacttcaacaacgtggaggaggccaaggaggccaccagcagaaagctgaagcacctgatcaccgactgcaagaacaacgagagagacatcagaagatacaagacccaggacatggtgatctacctgatggccagagacatcctgaaggacatcatccccgacagcgagaaggacaagtacgccaaggacagaaagctgctgctgaaggacgtgtgcgaggagggcttcctgagacaggccgtgaagatggagtacgagtacagcatcgaggagaagggcaagagaaccagaaccgtgaagatcacccaccccaacatgagcctgaagaactacggcgagttccacagactgctgaacgacgagagactgaagagcctgctgcagcagctggccaacatggacgagatcgactacaccgacctgatgggcgagttcgccgactacgaccagaagagaagcgagatcttcagactggcccagagcatcgagaagcacctgtacgagcagaacgagcagggcctgaacgacgagaagagcgacctgttctaccacaccagatacaacggcaagaagatccccagaagaaacagcttcagcagcctgctggagctgatcggcgaggaggagagccagatgaccgagacagacaagaagcagaccatcagcatcagaaacgccttcggccacaacacctacaaggtgagcctggccgagatgaacgccaccgagctgcccaacgtggccaagaccatcctgaagaagatggaggagctgagaaacaagctgacaggcggcggccccggcggcggcgccgccgccggcagcggcagccctaagaaaaaacgaaaagttggcagcggaagcaaaaggccggcggccacgaaaaaggccggccaggcaaaaaagaaaaagctcgagtacccatacgatgttccagattacgcttgagaattccccttgagcatctgacttctggctaataaaggaaatttattttcattgcaatagtgtgttggaattttttgtgtctctcaggtaccgagggcctatttcccatgattccttcatatttgcatatacgatacaaggctgttagagagataattggaattaatttgactgtaaacacaaagatattagtacaaaatacgtgacgtagaaagtaataatttcttgggtagtttgcagttttaaaattatgttttaaaatggactatcatatgcttaccgtaacttgaaagtatttcgatttcttggctttatatatcttgtggaaaggacgaaacaccggagaccacggcaggtctcagttgtagaagcctatcgttaggataggtatgacaactttttttgcggccgcaggaacccctagtgatggagttggccactccctctctgcgcgctcgctcgctcactgaggccgggcgaccaaaggtcgcccgacgcccgggctttgcccgggcggcctcagtgagcgagcgagcgcgcagctgcctgcaggggcgcctgatgcggtattttctccttacgcatctgtgcggtatttcacaccgcatacgtcaaagcaaccatagtacgcgccctgtagcggcgcattaagcgcggcgggtgtggtggttacgcgcagcgtgaccgctacacttgccagcgccttagcgcccgctcctttcgctttcttcccttcctttctcgccacgttcgccggctttccccgtcaagctctaaatcgggggctccctttagggttccgatttagtgctttacggcacctcgaccccaaaaaacttgatttgggtgatggttcacgtagtgggccatcgccctgatagacggtttttcgccctttgacgttggagtccacgttctttaatagtggactcttgttccaaactggaacaacactcaactctatctcgggctattcttttgatttataagggattttgccgatttcggtctattggttaaaaaatgagctgatttaacaaaaatttaacgcgaattttaacaaaatattaacgtttacaattttatggtgcactctcagtacaatctgctctgatgccgcatagttaagccagccccgacacccgccaacacccgctgacgcgccctgacgggcttgtctgctcccggcatccgcttacagacaagctgtgaccgtctccgggagctgcatgtgtcagaggttttcaccgtcatcaccgaaacgcgcgagacgaaagggcctcgtgatacgcctatttttataggttaatgtcatgataataatggtttcttagacgtcaggtggcacttttcggggaaatgtgcgcggaacccctatttgtttatttttctaaatacattcaaatatgtatccgctcatgagacaataaccctgataaatgcttcaataatattgaaaaaggaagagtatgagtattcaacatttccgtgtcgcccttattcccttttttgcggcattttgccttcctgtttttgctcacccagaaacgctggtgaaagtaaaagatgctgaagatcagttgggtgcacgagtgggttacatcgaactggatctcaacagcggtaagatccttgagagttttcgccccgaagaacgttttccaatgatgagcacttttaaagttctgctatgtggcgcggtattatcccgtattgacgccgggcaagagcaactcggtcgccgcatacactattctcagaatgacttggttgagtactcaccagtcacagaaaagcatcttacggatggcatgacagtaagagaattatgcagtgctgccataaccatgagtgataacactgcggccaacttacttctgacaacgatcggaggaccgaaggagctaaccgcttttttgcacaacatgggggatcatgtaactcgccttgatcgttgggaaccggagctgaatgaagccataccaaacgacgagcgtgacaccacgatgcctgtagcaatggcaacaacgttgcgcaaactattaactggcgaactacttactctagcttcccggcaacaattaatagactggatggaggcggataaagttgcaggaccacttctgcgctcggcccttccggctggctggtttattgctgataaatctggagccggtgagcgtggaagccgcggtatcattgcagcactggggccagatggtaagccctcccgtatcgtagttatctacacgacggggagtcaggcaactatggatgaacgaaatagacagatcgctgagataggtgcctcactgattaagcattggtaactgtcagaccaagtttactcatatatactttagattgatttaaaacttcatttttaatttaaaaggatctaggtgaagatcctttttgataatctcatgaccaaaatcccttaacgtgagttttcgttccactgagcgtcagaccccgtagaaaagatcaaaggatcttcttgagatcctttttttctgcgcgtaatctgctgcttgcaaacaaaaaaaccaccgctaccagcggtggtttgtttgccggatcaagagctaccaactctttttccgaaggtaactggcttcagcagagcgcagataccaaatactgttcttctagtgtagccgtagttaggccaccacttcaagaactctgtagcaccgcctacatacctcgctctgctaatcctgttaccagtggctgctgccagtggcgataagtcgtgtcttaccgggttggactcaagacgatagttaccggataaggcgcagcggtcgggctgaacggggggttcgtgcacacagcccagcttggagcgaacgacctacaccgaactgagatacctacagcgtgagctatgagaaagcgccacgcttcccgaagggagaaaggcggacaggtatccggtaagcggcagggtcggaacaggagagcgcacgagggagcttccagggggaaacgcctggtatctttatagtcctgtcgggtttcgccacctctgacttgagcgtcgatttttgtgatgctcgtcaggggggcggagcctatggaaaaacgccagcaacgcggcctttttacggttcctggccttttgctggccttttgctcacatgt

SEQ ID NO: 6 - DNA, 6793 bp, synthetic construct
  source 1..6793: mol_type = other DNA
cctgcaggcagctgcgcgctcgctcgctcactgaggccgcccgggcgtcgggcgacctttggtcgcccggcctcagtgagcgagcgagcgcgcagagagggagtggccaactccatcactaggggttcctgcggcctctagactcgaggcgttgacattgattattgactagttattaatagtaatcaattacggggtcattagttcatagcccatatatggagttccgcgttacataacttacggtaaatggcccgcctggctgaccgcccaacgacccccgcccattgacgtcaataatgacgtatgttcccatagtaacgccaatagggactttccattgacgtcaatgggtggagtatttacggtaaactgcccacttggcagtacatcaagtgtatcatatgccaagtacgccccctattgacgtcaatgacggtaaatggcccgcctggcattatgcccagtacatgaccttatgggactttcctacttggcagtacatctacgtattagtcatcgctattaccatggtgatgcggttttggcagtacatcaatgggcgtggatagcggtttgactcacggggatttccaagtctccaccccattgacgtcaatgggagtttgttttggcaccaaaatcaacgggactttccaaaatgtcgtaacaactccgccccattgacgcaaatgggcggtaggcgtgtacggtgggaggtctatataagcagagctctctggctaactaccggtgccaccatgccggcagctaagaaaaagaaactggatggcagcgtcgacatgagcaaggacaagaaaaccaaggccaagagaatgggcgtgaaggccctgctggcccacggcgaggacaagctgaccatgaccaccttcggcaagggcaacagaagcaagatcgagttcaccgagggctaccacggcagagccctggagacacccaagcacttcggcatcagaggcttcgaggtgagaagaatcgacgagaacgtggacctgtgcggcgacctggaggagggcaagaccatcgaggccctgctggtgaaccccagcgagaaggtgggcgaggactacctgaagctgaagggcaccctggagaagagattcttcggcagagagttcccccacgacaacatcagaatccagctgatctacaacatcctggacatctacaagatcctgggcatgaacgtggccgacatcctgtacgccctgggcaacatgcaggacaccgagctggacatcgacatgttcggccagagcctgaacaacgaggacaacctgaaggagtgcctgaagagaatgaggccctacatgggctacttcggcgacatcttcaagatcagccccaagggcgagaacatcgccgacagagagcacaacaagaaggtgctgagatgcatcagcgtgctgagaaacgccaccgcccacgacaagcaggacgagtacccctggttcaagagcagcgacatctacgagacaaagatcttcaaggccgacatgtggaagatcatcaaggaccagtacagagagaagatcaagaaggtgaacaaggacttcctgagcaagaacgccgtgaacatggccatcctgttcgacctgctgaacgccagagacgtggagcagaagaagcagatcaccgacgagttctacagattcaccatcagaaaggacggcaagaacctgggcatgaacctggtgaagatcagagagatcatcatcgacagatacgccagcggcctgagagacaagaagcacgacccccacagacagaagatcaacgtgatcgccgacttcctgatcttcagagccctgagccagaaccagggcatcatcgacaagaccgtgagcagcctgagactgaccaaggacgaggaggagaaggaccacgtgtaccagaacgccgccgagctggtgtggggcatggtgagcaactgcctgaccccctacttcaacgaccccaagaacaagtacatcctgaagtacaaggacgccaagacccccggcgacttcgaggactggatcaccagcaagatcagcgaggacgacggcgagcccttcgtgaaggtgctgagcttcctgtgcaacttcctggagggcaaggagatcaacgagctgctgaccgcctacatccacaagttcgagtgcatccaggacttcctgaacgtgatcagcagcctgggcgagaacgtgcagttccagcccagattcgccctgttcaacaacgccagcttcgcccagaacgtggccgtgcagctgagaatcctggccagcatcggcaagatgaagcccgacctgaccgaggccaagaggcccctgtacaaggccgccatcagaatgctgtgcccccccgagaagtgggagaagtacaccagcgacgagtggctggagaagaacatgctgctgaacagcgaggacagaaagaacgacaagaagaagaagcaggtgaaccccttcagaaacttcatcgccggcaacgtgatcgagagcagaagattcatgtacctggtgagatacagcaagcccaaggccgtgagagccatcatgcagaacagaagcatcgtgaactacgtgctgcacagactgcccagcgagcaggtgcacagatacgccagcgtgttccccgagaacttcgccgacctggagcaggagatcgacttcctgaccaagaagctgttcgagttcagcttcgaggagctgctgcacgagaaggacgtgatcctgaacaacagcagaagccacaagcccagcctggagatcgagagactgaaggccatcaccggcctgtacctgagcgtggcctacatcgccatcaagaacatcgtgaaggccaacgccagatactacatcgccttcgccgtgttcgagagagacaaggagctggtgaaggccaaggacgccagaatccagaccaagatccccgagacagacttccccgactacttctgcctgacccagtactacctggacagagacgaggagaagaagttccccggcgaccccagagacaaggaggccttcttcgagcacctgagaaagaccaagagacacttcagcaagcagtggagagagtggctgaacgagaagatcgccgacgccaagagcagccaggccaccggcctgctgctgagagaggccagaaacgacgtggagcacctgaacgtgctgagagccatccccgactacatccaggacttcagacacggcgagaagggcgagacagccatgaacagctacttcgagctgtaccactacctgatgcagagactgatgctgaagaacaccgagctggacctgagccactggagcggctggatcatgagaagcggcagacccgacagagacttgatccagatcgccttcgtgagcctggcctacaacctgcccagatacagaaacctgaccaaggagcaccacttcgacgacaccgtgctgcagaagatcagagagaaggagagcctggacacaggcggcggccccggcggcggcgccgccgccggcagcggcagccctaagaaaaaacgaaaagttggcagcggaagcaaaaggccggcggccacgaaaaaggccggccaggcaaaaaagaaaaagctcgagtacccatacgatgttccagattacgcttgagaattccccttgagcatctgacttctggctaataaaggaaatttattttcattgcaatagtgtgttggaattttttgtgtctctcaggtaccgagggcctatttcccatgattccttcatatttgcatatacgatacaaggctgttagagagataattggaattaatttgactgtaaacacaaagatattagtacaaaatacgtgacgtagaaagtaataatttcttgggtagtttgcagttttaaaattatgttttaaaatggactatcatatgcttaccgtaacttgaaagtatttcgatttcttggctttatatatcttgtggaaaggacgaaacaccggaagataactctacaaacctgtagggttctgagacggagaccacggcaggtctcattttttgcggccgcaggaacccctagtgatggagttggccactccctctctgcgcgctcgctcgctcactgaggccgggcgaccaaaggtcgcccgacgcccgggctttgcccgggcggcctcagtgagcgagcgagcgcgcagctgcctgcaggggcgcctgatgcggtattttctccttacgcatctgtgcggtatttcacaccgcatacgtcaaagcaaccatagtacgcgccctgtagcggcgcattaagcgcggcgggtgtggtggttacgcgcagcgtgaccgctacacttgccagcgccttagcgcccgctcctttcgctttcttcccttcctttctcgccacgttcgccggctttccccgtcaagctctaaatcgggggctccctttagggttccgatttagtgctttacggcacctcgaccccaaaaaacttgatttgggtgatggttcacgtagtgggccatcgccctgatagacggtttttcgccctttgacgttggagtccacgttctttaatagtggactcttgttccaaactggaacaacactcaactctatctcgggctattcttttgatttataagggattttgccgatttcggtctattggttaaaaaatgagctgatttaacaaaaatttaacgcgaattttaacaaaatattaacgtttacaattttatggtgcactctcagtacaatctgctctgatgccgcatagttaagccagccccgacacccgccaacacccgctgacgcgccctgacgggcttgtctgctcccggcatccgcttacagacaagctgtgaccgtctccgggagctgcatgtgtcagaggttttcaccgtcatcaccgaaacgcgcgagacgaaagggcctcgtgatacgcctatttttataggttaatgtcatgataataatggtttcttagacgtcaggtggcacttttcggggaaatgtgcgcggaacccctatttgtttatttttctaaatacattcaaatatgtatccgctcatgagacaataaccctgataaatgcttcaataatattgaaaaaggaagagtatgagtattcaacatttccgtgtcgcccttattcccttttttgcggcattttgccttcctgtttttgctcacccagaaacgctggtgaaagtaaaagatgctgaagatcagttgggtgcacgagtgggttacatcgaactggatctcaacagcggtaagatccttgagagttttcgccccgaagaacgttttccaatgatgagcacttttaaagttctgctatgtggcgcggtattatcccgtattgacgccgggcaagagcaactcggtcgccgcatacactattctcagaatgacttggttgagtactcaccagtcacagaaaagcatcttacggatggcatgacagtaagagaattatgcagtgctgccataaccatgagtgataacactgcggccaacttacttctgacaacgatcggaggaccgaaggagctaaccgcttttttgcacaacatgggggatcatgtaactcgccttgatcgttgggaaccggagctgaatgaagccataccaaacgacgagcgtgacaccacgatgcctgtagcaatggcaacaacgttgcgcaaactattaactggcgaactacttactctagcttcccggcaacaattaatagactggatggaggcggataaagttgcaggaccacttctgcgctcggcccttccggctggctggtttattgctgataaatctggagccggtgagcgtggaagccgcggtatcattgcagcactggggccagatggtaagccctcccgtatcgtagttatctacacgacggggagtcaggcaactatggatgaacgaaatagacagatcgctgagataggtgcctcactgattaagcattggtaactgtcagaccaagtttactcatatatactttagattgatttaaaacttcatttttaatttaaaaggatctaggtgaagatcctttttgataatctcatgaccaaaatcccttaacgtgagttttcgttccactgagcgtcagaccccgtagaaaagatcaaaggatcttcttgagatcctttttttctgcgcgtaatctgctgcttgcaaacaaaaaaaccaccgctaccagcggtggtttgtttgccggatcaagagctaccaactctttttccgaaggtaactggcttcagcagagcgcagataccaaatactgttcttctagtgtagccgtagttaggccaccacttcaagaactctgtagcaccgcctacatacctcgctctgctaatcctgttaccagtggctgctgccagtggcgataagtcgtgtcttaccgggttggactcaagacgatagttaccggataaggcgcagcggtcgggctgaacggggggttcgtgcacacagcccagcttggagcgaacgacctacaccgaactgagatacctacagcgtgagctatgagaaagcgccacgcttcccgaagggagaaaggcggacaggtatccggtaagcggcagggtcggaacaggagagcgcacgagggagcttccagggggaaacgcctggtatctttatagtcctgtcgggtttcgccacctctgacttgagcgtcgatttttgtgatgctcgtcaggggggcggagcctatggaaaaacgccagcaacgcggcctttttacggttcctggccttttgctggccttttgctcacatgt

SEQ ID NO: 7 - DNA, 20 bp, synthetic construct
  source 1..20: mol_type = other DNA
ggagaccacggcaggtctca

SEQ ID NO: 8 - DNA, 6436 bp, synthetic construct
  source 1..6436: mol_type = other DNA
cctgcaggcagctgcgcgctcgctcgctcactgaggccgcccgggcgtcgggcgacctttggtcgcccggcctcagtgagcgagcgagcgcgcagagagggagtggccaactccatcactaggggttcctgcggcctctagactcgaggcgttgacattgattattgactagttattaatagtaatcaattacggggtcattagttcatagcccatatatggagttccgcgttacataacttacggtaaatggcccgcctggctgaccgcccaacgacccccgcccattgacgtcaataatgacgtatgttcccatagtaacgccaatagggactttccattgacgtcaatgggtggagtatttacggtaaactgcccacttggcagtacatcaagtgtatcatatgccaagtacgccccctattgacgtcaatgacggtaaatggcccgcctggcattatgcccagtacatgaccttatgggactttcctacttggcagtacatctacgtattagtcatcgctattaccatggtgatgcggttttggcagtacatcaatgggcgtggatagcggtttgactcacggggatttccaagtctccaccccattgacgtcaatgggagtttgttttggcaccaaaatcaacgggactttccaaaatgtcgtaacaactccgccccattgacgcaaatgggcggtaggcgtgtacggtgggaggtctatataagcagagctctctggctaactaccggtgccaccatgccggcagctaagaaaaagaaactggatggcagcgtcgacgcccaggtgtccaaacagaccagcaagaaaagggaactgagcatcgatgagtaccagggtgctagaaagtggtgcttcacaatcgcctttaacaaagctctggtcaatagggataaaaacgatggcctcttcgtggagtccctgctgagacacgagaagtacagcaaacacgactggtacgacgaggataccagagccctgatcaagtgctccactcaggccgccaatgcaaaggccgaggctctgagaaattatttcagccactaccggcactcccccgggtgtctgaccttcactgcagaggatgagcttaggacaattatggagcgcgcctacgagagggccatttttgagtgtcggcgaagagaaactgaggtgatcatcgagtttccatctctgtttgaaggggaccgcatcacaaccgccggagtggtattttttgtgagtttcttcgtggaacggagagtgctggaccggctgtacggggcagttagtggcctgaagaagaacgaggggcagtacaagctgacaaggaaagctctgagcatgtactgtctgaaagattccagatttacaaaggcatgggataagagagtgctcctctttcgcgatatcctggcccagctgggcagaatcccagctgaggcttacgagtactaccacggcgaacagggcgacaaaaagagggccaacgacaatgagggcaccaaccccaaaaggcacaaggataagtttattgagtttgcactgcactacctggaggcccagcactctgagatctgctttggcagaaggcacatcgtgagagaggaagctggcgccggcgatgagcacaagaagcacagaaccaaagggaaggtggtggtggacttctccaagaaggatgaggatcagtcttactacatcagtaagaacaacgtgattgtgaggatcgataagaatgccggccctcgctcctaccgcatggggctcaatgaactgaagtacctggtcctgctctctctgcaggggaagggcgatgacgctatcgccaagctgtataggtatcggcagcatgtggagaacattctggacgtggtgaaggtgactgataaagataaccacgtgttcctgccaaggtttgtgctcgaacagcacggaatcggccggaaggccttcaagcagagaattgacgggcgcgtgaaacatgtgcgcggggtgtgggaaaagaagaaggccgccacaaacgagatgacgctgcacgagaaggcccgcgacatcctccagtacgtgaatgagaattgcactcgcagcttcaatcctggcgagtataacaggctgctggtgtgcctggtgggtaaagacgtggagaacttccaggccggcctgaagcggcttcagctggctgagagaattgacggccgggtgtattctatcttcgcccagacttctaccatcaatgaaatgcaccaggtggtgtgtgaccagatcctcaatcggctgtgtcgaattggggatcagaagctgtacgactatgtgggcctgggcaagaaagatgagatcgactataaacagaaagtggcttggttcaaagagcacatcagtatcagacgcggctttctgaggaagaaattctggtacgactctaaaaagggcttcgctaagctggtggaggagcacctggaatccggaggcggacagcgggatgtggggctggataagaaatactaccacatcgatgccatcgggagattcgagggcgccaatcctgctctgtacgaaaccctggccagggacaggctgtgcctgatgatggcccagtactttctgggctccgttcgcaaagagctgggaaacaaaattgtgtggagcaacgactccatagagctgccggtggagggatctgtcgggaatgaaaaatcgatcgtgttctctgtgagcgattatggaaaactgtacgtcctggacgatgccgagtttctgggtagaatctgtgagtattttatgccacatgaaaagggcaagatcagataccacaccgtgtatgaaaaggggttcagagcctacaacgacctgcagaaaaaatgcgtggaggccgtgctggcattcgaagagaaggtggtgaaggccaagaaaatgtctgagaaagagggagcccactacatcgactttcgcgagatcctggcccagaccatgtgcaaggaagctgaaaagacagccgtcaataaggtgaggagggccttctttcaccaccaccttaaattcgtgatcgacgaatttggcctgttcagcgatgtgatgaaaaaatacggcatcgagaaggagtggaagtttccagtgaaaacaggcggcggccccggcggcggcgccgccgccggcagcggcagccctaagaaaaaacgaaaagttggcagcggaagcaaaaggccggcggccacgaaaaaggccggccaggcaaaaaagaaaaagctcgagtacccatacgatgttccagattacgcttgagaattccccttgagcatctgacttctggctaataaaggaaatttattttcattgcaatagtgtgttggaattttttgtgtctctcaggtaccgagggcctatttcccatgattccttcatatttgcatatacgatacaaggctgttagagagataattggaattaatttgactgtaaacacaaagatattagtacaaaatacgtgacgtagaaagtaataatttcttgggtagtttgcagttttaaaattatgttttaaaatggactatcatatgcttaccgtaacttgaaagtatttcgatttcttggctttatatatcttgtggaaaggacgaaacaccggagaccacggcaggtctcagctggagcagcccccgatttgtggggtgattacagcttttttgcggccgcaggaacccctagtgatggagttggccactccctctctgcgcgctcgctcgctcactgaggccgggcgaccaaaggtcgcccgacgcccgggctttgcccgggcggcctcagtgagcgagcgagcgcgcagctgcctgcaggggcgcctgatgcggtattttctccttacgcatctgtgcggtatttcacaccgcatacgtcaaagcaaccatagtacgcgccctgtagcggcgcattaagcgcggcgggtgtggtggttacgcgcagcgtgaccgctacacttgccagcgccttagcgcccgctcctttcgctttcttcccttcctttctcgccacgttcgccggctttccccgtcaagctctaaatcgggggctccctttagggttccgatttagtgctttacggcacctcgaccccaaaaaacttgatttgggtgatggttcacgtagtgggccatcgccctgatagacggtttttcgccctttgacgttggagtccacgttctttaatagtggactcttgttccaaactggaacaacactcaactctatctcgggctattcttttgatttataagggattttgccgatttcggtctattggttaaaaaatgagctgatttaacaaaaatttaacgcgaattttaacaaaatattaacgtttacaattttatggtgcactctcagtacaatctgctctgatgccgcatagttaagccagccccgacacccgccaacacccgctgacgcgccctgacgggcttgtctgctcccggcatccgcttacagacaagctgtgaccgtctccgggagctgcatgtgtcagaggttttcaccgtcatcaccgaaacgcgcgagacgaaagggcctcgtgatacgcctatttttataggttaatgtcatgataataatggtttcttagacgtcaggtggcacttttcggggaaatgtgcgcggaacccctatttgtttatttttctaaatacattcaaatatgtatccgctcatgagacaataaccctgataaatgcttcaataatattgaaaaaggaagagtatgagtattcaacatttccgtgtcgcccttattcccttttttgcggcattttgccttcctgtttttgctcacccagaaacgctggtgaaagtaaaagatgctgaagatcagttgggtgcacgagtgggttacatcgaactggatctcaacagcggtaagatccttgagagttttcgccccgaagaacgttttccaatgatgagcacttttaaagttctgctatgtggcgcggtattatcccgtattgacgccgggcaagagcaactcggtcgccgcatacactattctcagaatgacttggttgagtactcaccagtcacagaaaagcatcttacggatggcatgacagtaagagaattatgcagtgctgccataaccatgagtgataacactgcggccaacttacttctgacaacgatcggaggaccgaaggagctaaccgcttttttgcacaacatgggggatcatgtaactcgccttgatcgttgggaaccggagctgaatgaagccataccaaacgacgagcgtgacaccacgatgcctgtagcaatggcaacaacgttgcgcaaactattaactggcgaactacttactctagcttcccggcaacaattaatagactggatggaggcggataaagttgcaggaccacttctgcgctcggcccttccggctggctggtttattgctgataaatctggagccggtgagcgtggaagccgcggtatcattgcagcactggggccagatggtaagccctcccgtatcgtagttatctacacgacggggagtcaggcaactatggatgaacgaaatagacagatcgctgagataggtgcctcactgattaagcattggtaactgtcagaccaagtttactcatatatactttagattgatttaaaacttcatttttaatttaaaaggatctaggtgaagatcctttttgataatctcatgaccaaaatcccttaacgtgagttttcgttccactgagcgtcagaccccgtagaaaagatcaaaggatcttcttgagatcctttttttctgcgcgtaatctgctgcttgcaaacaaaaaaaccaccgctaccagcggtggtttgtttgccggatcaagagctaccaactctttttccgaaggtaactggcttcagcagagcgcagataccaaatactgttcttctagtgtagccgtagttaggccaccacttcaagaactctgtagcaccgcctacatacctcgctctgctaatcctgttaccagtggctgctgccagtggcgataagtcgtgtcttaccgggttggactcaagacgatagttaccggataaggcgcagcggtcgggctgaacggggggttcgtgcacacagcccagcttggagcgaacgacctacaccgaactgagatacctacagcgtgagctatgagaaagcgccacgcttcccgaagggagaaaggcggacaggtatccggtaagcggcagggtcggaacaggagagcgcacgagggagcttccagggggaaacgcctggtatctttatagtcctgtcgggtttcgccacctctgacttgagcgtcgatttttgtgatgctcgtcaggggggcggagcctatggaaaaacgccagcaacgcggcctttttacggttcctggccttttgctggccttttgctcacatgt

SEQ ID NO: 9 - DNA, 30 bp, synthetic construct
  source 1..30: mol_type = other DNA
ggtactcctggaagatgtccaccagggtct

SEQ ID NO: 10 - DNA, 28 bp, synthetic construct
  source 1..28: mol_type = other DNA
ccactgcggccccctctcctcttccttc

SEQ ID NO: 11 - DNA, 23 bp, synthetic construct
  source 1..23: mol_type = other DNA
ggctggagcactgtctgcgcaca

SEQ ID NO: 12 - DNA, 25 bp, synthetic construct
  source 1..25: mol_type = other DNA
aagctcatctctcctatgtgctggc

SEQ ID NO: 13 - DNA, 29 bp, synthetic construct
  source 1..29: mol_type = other DNA
tgggtgcagcctgggaccacttggcatgg

SEQ ID NO: 14 - DNA, 24 bp, synthetic construct
  source 1..24: mol_type = other DNA
tctttctttggtctgcattcacat

SEQ ID NO: 15 - DNA, 25 bp, synthetic construct
  source 1..25: mol_type = other DNA
ggccttggtgaggtttgatccgcat

SEQ ID NO: 16 - DNA, 26 bp, synthetic construct
  source 1..26: mol_type = other DNA
acaaacaaatgctttctccgctctga

SEQ ID NO: 17 - DNA, 28 bp, synthetic construct
  source 1..28: mol_type = other DNA
gcaggaacatttacacgtctgcggatct

SEQ ID NO: 18 - DNA, 26 bp, synthetic construct
  source 1..26: mol_type = other DNA
agtacgttcgtttaactcaagctgcc

SEQ ID NO: 19 - DNA, 36 bp, synthetic construct
  source 1..36: mol_type = other DNA
gttgtagaagccgttcattcgggacggtatgacaac

SEQ ID NO: 20 - DNA, 36 bp, synthetic construct
  source 1..36: mol_type = other DNA
gttgtagaagcctatcgttaggataggtatgacaac

SEQ ID NO: 21 - DNA, 36 bp, synthetic construct
  source 1..36: mol_type = other DNA
ggaagataactctacaaacctgtagggttctgagac

SEQ ID NO: 22 - DNA, 20 bp, synthetic construct
  source 1..20: mol_type = other DNA
ccatggggaaggtgaaggtc

SEQ ID NO: 23 - DNA, 21 bp, synthetic construct
  source 1..21: mol_type = other DNA
gaaggggtcattgatggcaac

SEQ ID NO: 24 - DNA, 20 bp, synthetic construct
  source 1..20: mol_type = other DNA
acctccaccatgccaagtgg

SEQ ID NO: 25 - DNA, 20 bp, synthetic construct
  source 1..20: mol_type = other DNA
cagggtctcgattggatggc

SEQ ID NO: 26 - DNA, 20 bp, synthetic construct
  source 1..20: mol_type = other DNA
caatgacgagggcctggagt

SEQ ID NO: 27 - DNA, 20 bp, synthetic construct
  source 1..20: mol_type = other DNA
tctttggtctgcattcacat

SEQ ID NO: 28 - DNA, 7102 bp, synthetic construct
  source 1..7102: mol_type = other DNA
cctgcaggcagctgcgcgctcgctcgctcactgaggccgcccgggcgtcgggcgacctttggtcgcccggcctcagtgagcgagcgagcgcgcagagagggagtggccaactccatcactaggggttcctgcggcctctagactcgaggcgttgacattgattattgactagttattaatagtaatcaattacggggtcattagttcatagcccatatatggagttccgcgttacataacttacggtaaatggcccgcctggctgaccgcccaacgacccccgcccattgacgtcaataatgacgtatgttcccatagtaacgccaatagggactttccattgacgtcaatgggtggagtatttacggtaaactgcccacttggcagtacatcaagtgtatcatatgccaagtacgccccctattgacgtcaatgacggtaaatggcccgcctggcattatgcccagtacatgaccttatgggactttcctacttggcagtacatctacgtattagtcatcgctattaccatggtgatgcggttttggcagtacatcaatgggcgtggatagcggtttgactcacggggatttccaagtctccaccccattgacgtcaatgggagtttgttttggcaccaaaatcaacgggactttccaaaatgtcgtaacaactccgccccattgacgcaaatgggcggtaggcgtgtacggtgggaggtctatataagcagagctctctggctaactaccggtgccaccatgagccccaagaagaagagaaaggtggaggccagcatcgaaaaaaaaaagtccttcgccaagggcatgggcgtgaagtccacactcgtgtccggctccaaagtgtacatgacaaccttcgccgaaggcagcgacgccaggctggaaaagatcgtggagggcgacagcatcaggagcgtgaatgagggcgaggccttcagcgctgaaatggccgataaaaacgccggctataagatcggcaacgccaaattcagccatcctaagggctacgccgtggtggctaacaaccctctgtatacaggacccgtccagcaggatatgctcggcctgaaggaaactctggaaaagaggtacttcggcgagagcgctgatggcaatgacaatatttgtatccaggtgatccataacatcctggacattgaaaaaatcctcgccgaatacattaccaacgccgcctacgccgtcaacaatatctccggcctggataaggacattattggattcggcaagttctccacagtgtatacctacgacgaattcaaagaccccgagcaccatagggccgctttcaacaataacgataagctcatcaacgccatcaaggcccagtatgacgagttcgacaacttcctcgataaccccagactcggctatttcggccaggcctttttcagcaaggagggcagaaattacatcatcaattacggcaacgaatgctatgacattctggccctcctgagcggactgaggcactgggtggtccataacaacgaagaagagtccaggatctccaggacctggctctacaacctcgataagaacctcgacaacgaatacatctccaccctcaactacctctacgacaggatcaccaatgagctgaccaactccttctccaagaactccgccgccaacgtgaactatattgccgaaactctgggaatcaaccctgccgaattcgccgaacaatatttcagattcagcattatgaaagagcagaaaaacctcggattcaatatcaccaagctcagggaagtgatgctggacaggaaggatatgtccgagatcaggaaaaatcataaggtgttcgactccatcaggaccaaggtctacaccatgatggactttgtgatttataggtattacatcgaagaggatgccaaggtggctgccgccaataagtccctccccgataatgagaagtccctgagcgagaaggatatctttgtgattaacctgaggggctccttcaacgacgaccagaaggatgccctctactacgatgaagctaatagaatttggagaaagctcgaaaatatcatgcacaacatcaaggaatttaggggaaacaagacaagagagtataagaagaaggacgcccctagactgcccagaatcctgcccgctggccgtgatgtttccgccttcagcaaactcatgtatgccctgaccatgttcctggatggcaaggagatcaacgacctcctgaccaccctgattaataaattcgataacatccagagcttcctgaaggtgatgcctctcatcggagtcaacgctaagttcgtggaggaatacgcctttttcaaagactccgccaagatcgccgatgagctgaggctgatcaagtccttcgctagaatgggagaacctattgccgatgccaggagggccatgtatatcgacgccatccgtattttaggaaccaacctgtcctatgatgagctcaaggccctcgccgacaccttttccctggacgagaacggaaacaagctcaagaaaggcaagcacggcatgagaaatttcattattaataacgtgatcagcaataaaaggttccactacctgatcagatacggtgatcctgcccacctccatgagatcgccaaaaacgaggccgtggtgaagttcgtgctcggcaggatcgctgacatccagaaaaaacagggccagaacggcaagaaccagatcgacaggtactacgaaacttgtatcggaaaggataagggcaagagcgtgagcgaaaaggtggacgctctcacaaagatcatcaccggaatgaactacgaccaattcgacaagaaaaggagcgtcattgaggacaccggcagggaaaacgccgagagggagaagtttaaaaagatcatcagcctgtacctcaccgtgatctaccacatcctcaagaatattgtcaatatcaacgccaggtacgtcatcggattccattgcgtcgagcgtgatgctcaactgtacaaggagaaaggctacgacatcaatctcaagaaactggaagagaagggattcagctccgtcaccaagctctgcgctggcattgatgaaactgcccccgataagagaaaggacgtggaaaaggagatggctgaaagagccaaggagagcattgacagcctcgagagcgccaaccccaagctgtatgccaattacatcaaatacagcgacgagaagaaagccgaggagttcaccaggcagattaacagggagaaggccaaaaccgccctgaacgcctacctgaggaacaccaagtggaatgtgatcatcagggaggacctcctgagaattgacaacaagacatgtaccctgttcagaaacaaggccgtccacctggaagtggccaggtatgtccacgcctatatcaacgacattgccgaggtcaattcctacttccaactgtaccattacatcatgcagagaattatcatgaatgagaggtacgagaaaagcagcggaaaggtgtccgagtacttcgacgctgtgaatgacgagaagaagtacaacgataggctcctgaaactgctgtgtgtgcctttcggctactgtatccccaggtttaagaacctgagcatcgaggccctgttcgataggaacgaggccgccaagttcgacaaggagaaaaagaaggtgtccggcaattccggatccggacctaagaaaaagaggaaggtggcggccgcttacccatacgatgttccagattacgcttgaggtaccctagagctcgctgatcagcctcgactgtgccttctagttgccagccatctgttgtttgcccctcccccgtgccttccttgaccctggaaggtgccactcccactgtcctttcctaataaaatgaggaaattgcatcgcattgtctgagtaggtgtcattctattctggggggtggggtggggcaggacagcaagggggaggattgggaagagaatagcaggcatgctggggagagggcctatttcccatgattccttcatatttgcatatacgatacaaggctgttagagagataattggaattaatttgactgtaaacacaaagatattagtacaaaatacgtgacgtagaaagtaataatttcttgggtagtttgcagttttaaaattatgttttaaaatggactatcatatgcttaccgtaacttgaaagtatttcgatttcttggctttatatatcttgtggaaaggacgaaacaccgcaagtaaacccctaccaactggtcggggtttgaaacgggtcttcgagaagacctcaagtaaacccctaccaactggtcggggtttgaaactttttttcccgggaatggccgcaggaacccctagtgatggagttggccactccctctctgcgcgctcgctcgctcactgaggccgggcgaccaaaggtcgcccgacgcccgggctttgcccgggcggcctcagtgagcgagcgagcgcgcagctgcctgcaggggcgcctgatgcggtattttctccttacgcatctgtgcggtatttcacaccgcatacgtcaaagcaaccatagtacgcgccctgtagcggcgcattaagcgcggcgggtgtggtggttacgcgcagcgtgaccgctacacttgccagcgccctagcgcccgctcctttcgctttcttcccttcctttctcgccacgttcgccggctttccccgtcaagctctaaatcgggggctccctttagggttccgatttagtgctttacggcacctcgaccccaaaaaacttgatttgggtgatggttcacgtagtgggccatcgccctgatagacggtttttcgccctttgacgttggagtccacgttctttaatagtggactcttgttccaaactggaacaacactcaaccctatctcgggctattcttttgatttataagggattttgccgatttcggcctattggttaaaaaatgagctgatttaacaaaaatttaacgcgaattttaacaaaatattaacgtttacaattttatggtgcactctcagtacaatctgctctgatgccgcatagttaagccagccccgacacccgccaacacccgctgacgcgccctgacgggcttgtctgctcccggcatccgcttacagacaagctgtgaccgtctccgggagctgcatgtgtcagaggttttcaccgtcatcaccgaaacgcgcgagacgaaagggcctcgtgatacgcctatttttataggttaatgtcatgataataatggtttcttagacgtcaggtggcacttttcggggaaatgtgcgcggaacccctatttgtttatttttctaaatacattcaaatatgtatccgctcatgagacaataaccctgataaatgcttcaataatattgaaaaaggaagagtatgagtattcaacatttccgtgtcgcccttattcccttttttgcggcattttgccttcctgtttttgctcacccagaaacgctggtgaaagtaaaagatgctgaagatcagttgggtgcacgagtgggttacatcgaactggatctcaacagcggtaagatccttgagagttttcgccccgaagaacgttttccaatgatgagcacttttaaagttctgctatgtggcgcggtattatcccgtattgacgccgggcaagagcaactcggtcgccgcatacactattctcagaatgacttggttgagtactcaccagtcacagaaaagcatcttacggatggcatgacagtaagagaattatgcagtgctgccataaccatgagtgataacactgcggccaacttacttctgacaacgatcggaggaccgaaggagctaaccgcttttttgcacaacatgggggatcatgtaactcgccttgatcgttgggaaccggagctgaatgaagccataccaaacgacgagcgtgacaccacgatgcctgtagcaatggcaacaacgttgcgcaaactattaactggcgaactacttactctagcttcccggcaacaattaatagactggatggaggcggataaagttgcaggaccacttctgcgctcggcccttccggctggctggtttattgctgataaatctggagccggtgagcgtggaagccgcggtatcattgcagcactggggccagatggtaagccctcccgtatcgtagttatctacacgacggggagtcaggcaactatggatgaacgaaatagacagatcgctgagataggtgcctcactgattaagcattggtaactgtcagaccaagtttactcatatatactttagattgatttaaaacttcatttttaatttaaaaggatctaggtgaagatcctttttgataatctcatgaccaaaatcccttaacgtgagttttcgttccactgagcgtcagaccccgtagaaaagatcaaaggatcttcttgagatcctttttttctgcgcgtaatctgctgcttgcaaacaaaaaaaccaccgctaccagcggtggtttgtttgccggatcaagagctaccaactctttttccgaaggtaactggcttcagcagagcgcagataccaaatactgtccttctagtgtagccgtagttaggccaccacttcaagaactctgtagcaccgcctacatacctcgctctgctaatcctgttaccagtggctgctgccagtggcgataagtcgtgtcttaccgggttggactcaagacgatagttaccggataaggcgcagcggtcgggctgaacggggggttcgtgcacacagcccagcttggagcgaacgacctacaccgaactgagatacctacagcgtgagctatgagaaagcgccacgcttcccgaagggagaaaggcggacaggtatccggtaagcggcagggtcggaacaggagagcgcacgagggagcttccagggggaaacgcctggtatctttatagtcctgtcgggtttcgccacctctgacttgagcgtcgatttttgtgatgctcgtcaggggggcggagcctatggaaaaacgccagcaacgcggcctttttacggttcctggccttttgctggccttttgctcacatgt

SEQ ID NO: 29 - DNA, 29 bp, synthetic construct
  source 1..29: mol_type = other DNA
gcagcctgggaccacttggcatggtggag

SEQ ID NO: 30 - DNA, 30 bp, synthetic construct
  source 1..30: mol_type = other DNA
cctggaagatgtccaccagggtctcgattg

SEQ ID NO: 31 - DNA, 30 bp, synthetic construct
  source 1..30: mol_type = other DNA
atgttggactcctcagtgggcacacactcc

SEQ ID NO: 32 - DNA, 96 bp, synthetic construct
  source 1..96: mol_type = other DNA
cctggaagatgtccaccagggtctcgattgcaagtaaacccctaccaactggtcggggtttgaaacatgttggactcctcagtgggcacacactcc

SEQ ID NO: 33 - DNA, 30 bp, synthetic construct
  source 1..30: mol_type = other DNA
gtgctgtaggaagctcatctctcctatgtg

SEQ ID NO: 34 - DNA, 30 bp, synthetic construct; identical to SEQ ID NO: 9
  source 1..30: mol_type = other DNA

SEQ ID NO: 35 - DNA, 96 bp, synthetic construct
  source 1..96: mol_type = other DNA
ggtactcctggaagatgtccaccagggtctcaagtaaacccctaccaactggtcggggtttgaaacgtgctgtaggaagctcatctctcctatgtg

SEQ ID NO: 36 - DNA, 20 bp, synthetic construct
  source 1..20: mol_type = other DNA
cttcaagccgtcctgtgtgc

SEQ ID NO: 37 - DNA, 20 bp, synthetic construct
  source 1..20: mol_type = other DNA
gctcatctctcctatgtgct

SEQ ID NO: 38 - DNA, 22 bp, synthetic construct
  source 1..22: mol_type = other DNA
gctgagtatgtcgtggagtcta

SEQ ID NO: 39 - DNA, 20 bp, synthetic construct
  source 1..20: mol_type = other DNA
gtggttcacacccatcacaa

SEQ ID NO: 40 - DNA, 25 bp, synthetic construct
  source 1..25: mol_type = other DNA
tgcacccaagacagcagaaagttca

SEQ ID NO: 41 - DNA, 25 bp, synthetic construct
  source 1..25: mol_type = other DNA
aaggctccaatgcacccaagacagc

SEQ ID NO: 42 - DNA, 25 bp, synthetic construct
  source 1..25: mol_type = other DNA
tggaggtagagcagcaaggcaaggc

SEQ ID NO: 43 - DNA, 25 bp, synthetic construct
  source 1..25: mol_type = other DNA
ccctcctccttctgccatgggtgca

SEQ ID NO: 44 - DNA, 25 bp, synthetic construct
  source 1..25: mol_type = other DNA
catccatgaacttcaccacttcgtg

SEQ ID NO: 45 - DNA, 25 bp, synthetic construct
  source 1..25: mol_type = other DNA
gtagctgcgctgatagacatccatg

SEQ ID NO: 46 - DNA, 25 bp, synthetic construct
  source 1..25: mol_type = other DNA
atggcttgaagatgtactcgatctc

SEQ ID NO: 47 - DNA, 25 bp, synthetic construct
  source 1..25: mol_type = other DNA
catcaggggcacacaggatggcttg

SEQ ID NO: 48 - DNA, 25 bp, synthetic construct
  source 1..25: mol_type = other DNA
agcagcccccgcatcgcatcagggg

SEQ ID NO: 49 - DNA, 25 bp, synthetic construct
  source 1..25: mol_type = other DNA
ttgcagcagcccccgcatcgcatca

SEQ ID NO: 50 - DNA, 25 bp, synthetic construct
  source 1..25: mol_type = other DNA
tcgtcattgcagcagcccccgcatc

SEQ ID NO: 51 - DNA, 25 bp, synthetic construct
  source 1..25: mol_type = other DNA
actccaggccctcgtcattgcagca

SEQ ID NO: 52 - DNA, 25 bp, synthetic construct
  source 1..25: mol_type = other DNA
cacacactccaggccctcgtcattg

SEQ ID NO: 53 - DNA, 25 bp, synthetic construct
  source 1..25: mol_type = other DNA
tgggcacacactccaggccctcgtc

SEQ ID NO: 54 - DNA, 25 bp, synthetic construct
  source 1..25: mol_type = other DNA
ctcagtgggcacacactccaggccc

SEQ ID NO: 55 - DNA, 25 bp, synthetic construct
  source 1..25: mol_type = other DNA
tgcatggtgatgttggactcctcag

SEQ ID NO: 56 - DNA, 25 bp, synthetic construct
  source 1..25: mol_type = other DNA
atctgcatggtgatgttggactcct

SEQ ID NO: 57 - DNA, 25 bp, synthetic construct
  source 1..25: mol_type = other DNA
gcataatctgcatggtgatgttgga

SEQ ID NO: 58 - DNA, 25 bp, synthetic construct
  source 1..25: mol_type = other DNA
tccgcataatctgcatggtgatgtt

SEQ ID NO: 59 - DNA, 25 bp, synthetic construct
  source 1..25: mol_type = other DNA
tgtgctggccttggtgaggtttgat

SEQ ID NO: 60 - DNA, 25 bp, synthetic construct
  source 1..25: mol_type = other DNA
ttcacatttgttgtgctgtaggaag

SEQ ID NO: 61 - DNA, 25 bp, synthetic construct
  source 1..25: mol_type = other DNA
gtctgcattcacatttgttgtgctg

SEQ ID NO: 62 - DNA, 26 bp, synthetic construct
  source 1..26: mol_type = other DNA
gggcacgaccgcttaccttggcatgg

SEQ ID NO: 63 - DNA, 25 bp, synthetic construct
  source 1..25: mol_type = other DNA
gcgccagcagggcacgaccgcttac

SEQ ID NO: 64 - DNA, 26 bp, synthetic construct
  source 1..26: mol_type = other DNA
tgcagcctgggaccactgaggacaga

SEQ ID NO: 65 - DNA, 26 bp, synthetic construct
  source 1..26: mol_type = other DNA
ctgaggacagaaagagagcaaggcat

SEQ ID NO: 66 - DNA, 25 bp, synthetic construct
  source 1..25: mol_type = other DNA
ccactgaggacagaaagagagcaag

SEQ ID NO: 67 - DNA, 26 bp, synthetic construct
  source 1..26: mol_type = other DNA
cccatccaacagccagggggactcac

SEQ ID NO: 68 - DNA, 26 bp, synthetic construct
  source 1..26: mol_type = other DNA
tgaacttcaccactgcatgagaggcg

SEQ ID NO: 69 - DNA, 26 bp, synthetic construct
  source 1..26: mol_type = other DNA
ctgcatgagaggcgatgacacatgag

SEQ ID NO: 70 - DNA, 26 bp, synthetic construct
  source 1..26: mol_type = other DNA
caaagatgcccacctgcatggtgatg

SEQ ID NO: 71 - DNA, 26 bp, synthetic construct
  source 1..26: mol_type = other DNA
ttgccccacttcccaaagatgcccac

SEQ ID NO: 72 - DNA, 26 bp, synthetic construct
  source 1..26: mol_type = other DNA
ggtttgatccgcataatctggaaagg

SEQ ID NO: 73 - DNA, 26 bp, synthetic construct
  source 1..26: mol_type = other DNA
gactacatcctcacctgcattcacat

SEQ ID NO: 74 - DNA, 26 bp, synthetic construct
  source 1..26: mol_type = other DNA
taatgaatccgtgactacatcctcac

SEQ ID NO: 75 - DNA, 30 bp, synthetic construct
  source 1..30: mol_type = other DNA
tcgtcattgcagcagcccccgcatcgcatc

SEQ ID NO: 76 - DNA, 30 bp, synthetic construct
  source 1..30: mol_type = other DNA
atagacatccatgaacttcaccacttcgtg

SEQ ID NO: 77 - DNA, 30 bp, synthetic construct
  source 1..30: mol_type = other DNA
aagatgtccaccagggtctcgattggatgg

SEQ ID NO: 78 - DNA, 30 bp, synthetic construct
  source 1..30: mol_type = other DNA
cgtcattgcagcagcccccgcatcgcatca

SEQ ID NO: 79 - DNA, 30 bp, synthetic construct
  source 1..30: mol_type = other DNA
tagacatccatgaacttcaccacttcgtga

SEQ ID NO: 80 - DNA, 30 bp, synthetic construct
  source 1..30: mol_type = other DNA
tttgatccgcataatctgcatggtgatgtt

SEQ ID NO: 81 - DNA, 30 bp, synthetic construct
  source 1..30: mol_type = other DNA
agacatccatgaacttcaccacttcgtgat

SEQ ID NO: 82 - DNA, 30 bp, synthetic construct
  source 1..30: mol_type = other DNA
acatccatgaacttcaccacttcgtgatga

SEQ ID NO: 83 - DNA, 30 bp, synthetic construct
  source 1..30: mol_type = other DNA
ccctcgtcattgcagcagcccccgcatcgc

SEQ ID NO: 84 - DNA, 30 bp, synthetic construct
  source 1..30: mol_type = other DNA
gccctcgtcattgcagcagcccccgcatcg

SEQ ID NO: 85 - DNA, 30 bp, synthetic construct; identical to SEQ ID NO: 31
  source 1..30: mol_type = other DNA

SEQ ID NO: 86 - DNA, 30 bp, synthetic construct
  source 1..30: mol_type = other DNA
tgttggactcctcagtgggcacacactcca

SEQ ID NO: 87 - DNA, 30 bp, synthetic construct
  source 1..30: mol_type = other DNA
ccaatgcacccaagacagcagaaagttcat

SEQ ID NO: 88 - DNA, 30 bp, synthetic construct
  source 1..30: mol_type = other DNA
tccaatgcacccaagacagcagaaagttca

SEQ ID NO: 89 - DNA, 30 bp, synthetic construct
  source 1..30: mol_type = other DNA
ctccaatgcacccaagacagcagaaagttc

SEQ ID NO: 90 - DNA, 30 bp, synthetic construct
  source 1..30: mol_type = other DNA
cacacactccaggccctcgtcattgcagca

SEQ ID NO: 91 - DNA, 30 bp, synthetic construct
  source 1..30: mol_type = other DNA
gcacacactccaggccctcgtcattgcagc

SEQ ID NO: 92 - DNA, 30 bp, synthetic construct
  source 1..30: mol_type = other DNA
cacttcgtgatgattctgccctcctccttc

SEQ ID NO: 93 - DNA, 30 bp, synthetic construct
  source 1..30: mol_type = other DNA
ccacttcgtgatgattctgccctcctcctt

SEQ ID NO: 94 - DNA, 27 bp, synthetic construct
  source 1..27: mol_type = other DNA
ccttggtgaggtttgatccgcataatc

SEQ ID NO: 95 - DNA, 27 bp, synthetic construct
  source 1..27: mol_type = other DNA
aagatgtactcgatctcatcagggtac

SEQ ID NO: 96 - DNA, 27 bp, synthetic construct
  source 1..27: mol_type = other DNA
tttgatccgcataatctgcatggtgat

SEQ ID NO: 97 - DNA, 27 bp, synthetic construct
  source 1..27: mol_type = other DNA
tcgtcattgcagcagcccccgcatcgc

SEQ ID NO: 98 - DNA, 27 bp, synthetic construct
  source 1..27: mol_type = other DNA
aagatgtccaccagggtctcgattgga

SEQ ID NO: 99 - DNA, 27 bp, synthetic construct
  source 1..27: mol_type = other DNA
atgttggactcctcagtgggcacacac

SEQ ID NO: 100 - DNA, 27 bp, synthetic construct
  source 1..27: mol_type = other DNA
cgtcattgcagcagcccccgcatcgca

SEQ ID NO: 101 - DNA, 27 bp, synthetic construct
  source 1..27: mol_type = other DNA
tagacatccatgaacttcaccacttcg

SEQ ID NO: 102 - DNA, 27 bp, synthetic construct
  source 1..27: mol_type = other DNA
agacatccatgaacttcaccacttcgt

SEQ ID NO: 103 - DNA, 27 bp, synthetic construct
  source 1..27: mol_type = other DNA
acatccatgaacttcaccacttcgtga

SEQ ID NO: 104 - DNA, 27 bp, synthetic construct
  source 1..27: mol_type = other DNA
gacatccatgaacttcaccacttcgtg

SEQ ID NO: 105 - DNA, 27 bp, synthetic construct
  source 1..27: mol_type = other DNA
gcattcacatttgttgtgctgtaggaa

SEQ ID NO: 106 - DNA, 27 bp, synthetic construct
  source 1..27: mol_type = other DNA
atagacatccatgaacttcaccacttc

SEQ ID NO: 107 - DNA, 27 bp, synthetic construct
  source 1..27: mol_type = other DNA
gcacacactccaggccctcgtcattgc

SEQ ID NO: 108 - DNA, 27 bp, synthetic construct
  source 1..27: mol_type = other DNA
ccctcgtcattgcagcagcccccgcat

SEQ ID NO: 109 - DNA, 25 bp, synthetic construct
  source 1..25: mol_type = other DNA
ccttggtgaggtttgatccgcataa

SEQ ID NO: 110 - DNA, 27 bp, synthetic construct
  source 1..27: mol_type = other DNA
cacttcgtgatgattctgccctcctcc

SEQ ID NO: 111 - DNA, 27 bp, synthetic construct
  source 1..27: mol_type = other DNA
ccaatgcacccaagacagcagaaagtt

SEQ ID NO: 112 - DNA, 25 bp, synthetic construct
  source 1..25: mol_type = other DNA
agatgtactcgatctcatcagggta

SEQ ID NO: 113 - DNA, 27 bp, synthetic construct
  source 1..27: mol_type = other DNA
tccaatgcacccaagacagcagaaagt

SEQ ID NO: 114 - DNA, 25 bp, synthetic construct
  source 1..25: mol_type = other DNA
tttgatccgcataatctgcatggtg

SEQ ID NO: 115 - DNA, 27 bp, synthetic construct
  source 1..27: mol_type = other DNA
tggactcctcagtgggcacacactcca

SEQ ID NO: 116 - DNA, 25 bp, synthetic construct
  source 1..25: mol_type = other DNA
aagatgtccaccagggtctcgattg

SEQ ID NO: 117 - DNA, 25 bp, synthetic construct
  source 1..25: mol_type = other DNA
cgtcattgcagcagcccccgcatcg

SEQ ID NO: 118 - DNA, 25 bp, synthetic construct
  source 1..25: mol_type = other DNA
tcgtcattgcagcagcccccgcatc

SEQ ID NO: 119 - DNA, 25 bp, synthetic construct
  source 1..25: mol_type = other DNA
acatccatgaacttcaccacttcgt

SEQ ID NO: 120 - DNA, 25 bp, synthetic construct
  source 1..25: mol_type = other DNA
catccatgaacttcaccacttcgtg

SEQ ID NO: 121 - DNA, 25 bp, synthetic construct
  source 1..25: mol_type = other DNA
gcattcacatttgttgtgctgtagg

SEQ ID NO: 122 - DNA, 25 bp, synthetic construct
  source 1..25: mol_type = other DNA
atagacatccatgaacttcaccact

SEQ ID NO: 123 - DNA, 25 bp, synthetic construct
  source 1..25: mol_type = other DNA
gttggactcctcagtgggcacacac

SEQ ID NO: 124 - DNA, 25 bp, synthetic construct
  source 1..25: mol_type = other DNA
gacatccatgaacttcaccacttcg

SEQ ID NO: 125 - DNA, 25 bp, synthetic construct
  source 1..25: mol_type = other DNA
atgttggactcctcagtgggcacac

SEQ ID NO: 126 - DNA, 25 bp, synthetic construct
  source 1..25: mol_type = other DNA
tagacatccatgaacttcaccactt

SEQ ID NO: 127 - DNA, 25 bp, synthetic construct
  source 1..25: mol_type = other DNA
agacatccatgaacttcaccacttc

SEQ ID NO: 128 - DNA, 25 bp, synthetic construct
  source 1..25: mol_type = other DNA
tggactcctcagtgggcacacactc

SEQ ID NO: 129 - DNA, 25 bp, synthetic construct
  source 1..25: mol_type = other DNA
ccaatgcacccaagacagcagaaag

SEQ ID NO: 130 - DNA, 25 bp, synthetic construct
  source 1..25: mol_type = other DNA
tccaatgcacccaagacagcagaaa

SEQ ID NO: 131 - DNA, 25 bp, synthetic construct
  source 1..25: mol_type = other DNA
ccctcgtcattgcagcagcccccgc

SEQ ID NO: 132 - DNA, 30 bp, synthetic construct
  source 1..30: mol_type = other DNA
gacatccatgaacttcaccacttcgtgatg

SEQ ID NO: 133 - DNA, 30 bp, synthetic construct
  source 1..30: mol_type = other DNA
gcattcacatttgttgtgctgtaggaagct

SEQ ID NO: 134 - DNA, 30 bp, synthetic construct
  source 1..30: mol_type = other DNA
caccacttcgtgatgattctgccctcctcc

SEQ ID NO: 135 - DNA, 30 bp, synthetic construct
  source 1..30: mol_type = other DNA
ccttggtgaggtttgatccgcataatctgc

SEQ ID NO: 136 - DNA, 30 bp, synthetic construct
  source 1..30: mol_type = other DNA
caggccctcgtcattgcagcagcccccgca

SEQ ID NO: 137 - DNA, 30 bp, synthetic construct
  source 1..30: mol_type = other DNA
gcaaggctccaatgcacccaagacagcaga

SEQ ID NO: 138 - DNA, 30 bp, synthetic construct
  source 1..30: mol_type = other DNA
accacttcgtgatgattctgccctcctcct

SEQ ID NO: 139 - DNA, 30 bp, synthetic construct
  source 1..30: mol_type = other DNA
gctccaatgcacccaagacagcagaaagtt

SEQ ID NO: 140 - DNA, 30 bp, synthetic construct
  source 1..30: mol_type = other DNA
aagatgtactcgatctcatcagggtactcc

SEQ ID NO: 141 - DNA, 30 bp, synthetic construct
  source 1..30: mol_type = other DNA
cctcgtcattgcagcagcccccgcatcgca

SEQ ID NO: 142 - DNA, 30 bp, synthetic construct
  source 1..30: mol_type = other DNA
gttggactcctcagtgggcacacactccag

SEQ ID NO: 143 - DNA, 30 bp, synthetic construct
  source 1..30: mol_type = other DNA
cgcatcgcatcaggggcacacaggatggct

SEQ ID NO: 144 - DNA, 30 bp, synthetic construct
  source 1..30: mol_type = other DNA
gtagctgcgctgatagacatccatgaactt

SEQ ID NO: 145 - DNA, 30 bp, synthetic construct
  source 1..30: mol_type = other DNA
gaagatgtccaccagggtctcgattggatg

SEQ ID NO: 146 - DNA, 30 bp, synthetic construct
  source 1..30: mol_type = other DNA
aggctccaatgcacccaagacagcagaaag

SEQ ID NO: 147 - DNA, 30 bp, synthetic construct
  source 1..30: mol_type = other DNA
ggcaaggctccaatgcacccaagacagcag

SEQ ID NO: 148 - DNA, 27 bp, synthetic construct
  source 1..27: mol_type = other DNA
gccctcgtcattgcagcagcccccgca

SEQ ID NO: 149 - DNA, 27 bp, synthetic construct
  source 1..27: mol_type = other DNA
cgcatcgcatcaggggcacacaggatg

SEQ ID NO: 150 - DNA, 27 bp, synthetic construct
  source 1..27: mol_type = other DNA
ccacttcgtgatgattctgccctcctc

SEQ ID NO: 151 - DNA, 27 bp, synthetic construct
  source 1..27: mol_type = other DNA
acttcgtgatgattctgccctcctcct

SEQ ID NO: 152 - DNA, 27 bp, synthetic construct
  source 1..27: mol_type = other DNA
ctccaatgcacccaagacagcagaaag

SEQ ID NO: 153 - DNA, 27 bp, synthetic construct
  source 1..27: mol_type = other DNA
ccgcatcgcatcaggggcacacaggat

SEQ ID NO: 154 - DNA, 27 bp, synthetic construct
  source 1..27: mol_type = other DNA
catccatgaacttcaccacttcgtgat

SEQ ID NO: 155 - DNA, 27 bp, synthetic construct
  source 1..27: mol_type = other DNA
agatgtactcgatctcatcagggtact

SEQ ID NO: 156 - DNA, 27 bp, synthetic construct
  source 1..27: mol_type = other DNA
cacacactccaggccctcgtcattgca

SEQ ID NO: 157 - DNA, 27 bp, synthetic construct
  source 1..27: mol_type = other DNA
ttggactcctcagtgggcacacactcc

SEQ ID NO: 158 - DNA, 27 bp, synthetic construct
  source 1..27: mol_type = other DNA
tgttggactcctcagtgggcacacact

SEQ ID NO: 159 - DNA, 27 bp, synthetic construct
  source 1..27: mol_type = other DNA
gtagctgcgctgatagacatccatgaa

SEQ ID NO: 160 - DNA, 27 bp, synthetic construct
  source 1..27: mol_type = other DNA
gttggactcctcagtgggcacacactc

SEQ ID NO: 161 - DNA, 27 bp, synthetic construct
  source 1..27: mol_type = other DNA
caccacttcgtgatgattctgccctcc

SEQ ID NO: 162 - DNA, 27 bp, synthetic construct
  source 1..27: mol_type = other DNA
tagctgcgctgatagacatccatgaac

SEQ ID NO: 163 - DNA, 27 bp, synthetic construct
  source 1..27: mol_type = other DNA
gctccaatgcacccaagacagcagaaa

SEQ ID NO: 164 - DNA, 27 bp, synthetic construct
  source 1..27: mol_type = other DNA
ggactcctcagtgggcacacactccag

SEQ ID NO: 165 - DNA, 27 bp, synthetic construct
  source 1..27: mol_type = other DNA
atctgcatggtgatgttggactcctca

SEQ ID NO: 166 - DNA, 27 bp, synthetic construct
  source 1..27: mol_type = other DNA
agtagctgcgctgatagacatccatga

SEQ ID NO: 167 - DNA, 27 bp, synthetic construct
  source 1..27: mol_type = other DNA
accacttcgtgatgattctgccctcct

SEQ ID NO: 168 - DNA, 27 bp, synthetic construct
  source 1..27: mol_type = other DNA
gaagatgtccaccagggtctcgattgg

SEQ ID NO: 169 - DNA, 27 bp, synthetic construct
  source 1..27: mol_type = other DNA
aatgcacccaagacagcagaaagttca

SEQ ID NO: 170 - DNA, 27 bp, synthetic construct
  source 1..27: mol_type = other DNA
atgcacccaagacagcagaaagttcat

SEQ ID NO: 171 - DNA, 27 bp, synthetic construct
  source 1..27: mol_type = other DNA
gcttgaagatgtactcgatctcatcag

SEQ ID NO: 172 - DNA, 27 bp, synthetic construct
  source 1..27: mol_type = other DNA
ctgcattcacatttgttgtgctgtagg

SEQ ID NO: 173 - DNA, 27 bp, synthetic construct
  source 1..27: mol_type = other DNA
tctgcatggtgatgttggactcctcag

SEQ ID NO: 174 - DNA, 27 bp, synthetic construct
  source 1..27: mol_type = other DNA
caggccctcgtcattgcagcagccccc

SEQ ID NO: 175 - DNA, 27 bp, synthetic construct
  source 1..27: mol_type = other DNA
cttcgtgatgattctgccctcctcctt

SEQ ID NO: 176 - DNA, 27 bp, synthetic construct
  source 1..27: mol_type = other DNA
ctgcatggtgatgttggactcctcagt

SEQ ID NO: 177 - DNA, 27 bp, synthetic construct
  source 1..27: mol_type = other DNA
gcaaggctccaatgcacccaagacagc

SEQ ID NO: 178 - DNA, 27 bp, synthetic construct
  source 1..27: mol_type = other DNA
ggctccaatgcacccaagacagcagaa

SEQ ID NO: 179 - DNA, 25 bp, synthetic construct
  source 1..25: mol_type = other DNA
gccctcgtcattgcagcagcccccg

SEQ ID NO: 180 - DNA, 25 bp, synthetic construct
  source 1..25: mol_type = other DNA
gaagatgtccaccagggtctcgatt

SEQ ID NO: 181 - DNA, 25 bp, synthetic construct
  source 1..25: mol_type = other DNA
cgcatcgcatcaggggcacacagga

SEQ ID NO: 182 - DNA, 25 bp, synthetic construct
  source 1..25: mol_type = other DNA
gcacacactccaggccctcgtcatt

SEQ ID NO: 183 - DNA, 25 bp, synthetic construct
  source 1..25: mol_type = other DNA
cacttcgtgatgattctgccctcct

SEQ ID NO: 184 - DNA, 25 bp, synthetic construct
  source 1..25: mol_type = other DNA
ccacttcgtgatgattctgccctcc

SEQ ID NO: 185 - DNA, 25 bp, synthetic construct
  source 1..25: mol_type = other DNA
aagatgtactcgatctcatcagggt

SEQ ID NO: 186 - DNA, 25 bp, synthetic construct
  source 1..25: mol_type = other DNA
atttgttgtgctgtaggaagctcat

SEQ ID NO: 187 - DNA, 25 bp, synthetic construct
  source 1..25: mol_type = other DNA
ttggactcctcagtgggcacacact

SEQ ID NO: 188 - DNA, 25 bp, synthetic construct
  source 1..25: mol_type = other DNA
cacacactccaggccctcgtcattg

SEQ ID NO: 189 - DNA, 25 bp, synthetic construct
  source 1..25: mol_type = other DNA
ctccaatgcacccaagacagcagaa

SEQ ID NO: 190 - DNA, 25 bp, synthetic construct
  source 1..25: mol_type = other DNA
tgttggactcctcagtgggcacaca

SEQ ID NO: 191 - DNA, 25 bp, synthetic construct
  source 1..25: mol_type = other DNA
ctgcattcacatttgttgtgctgta

SEQ ID NO: 192 - DNA, 25 bp, synthetic construct
  source 1..25: mol_type = other DNA
acttcgtgatgattctgccctcctc

SEQ ID NO: 193 - DNA, 25 bp, synthetic construct
  source 1..25: mol_type = other DNA
gtagctgcgctgatagacatccatg

SEQ ID NO: 194 - DNA, 25 bp, synthetic construct
  source 1..25: mol_type = other DNA
aatgcacccaagacagcagaaagtt

SEQ ID NO: 195 - DNA, 25 bp, synthetic construct
  source 1..25: mol_type = other DNA
caccacttcgtgatgattctgccct

SEQ ID NO: 196 - DNA, 25 bp, synthetic construct
  source 1..25: mol_type = other DNA
cctcgtcattgcagcagcccccgca

SEQ ID NO: 197 - DNA, 25 bp, synthetic construct
  source 1..25: mol_type = other DNA
caatgcacccaagacagcagaaagt

SEQ ID NO: 198 - DNA, 25 bp, synthetic construct
  source 1..25: mol_type = other DNA
gcatcgcatcaggggcacacaggat

SEQ ID NO: 199 - DNA, 25 bp, synthetic construct
  source 1..25: mol_type = other DNA
ctgcatggtgatgttggactcctca

SEQ ID NO: 200 - DNA, 25 bp, synthetic construct
  source 1..25: mol_type = other DNA
ggactcctcagtgggcacacactcc

SEQ ID NO: 201 - DNA, 25 bp, synthetic construct
  source 1..25: mol_type = other DNA
tagctgcgctgatagacatccatga

SEQ ID NO: 202 - DNA, 25 bp, synthetic construct
  source 1..25: mol_type = other DNA
accacttcgtgatgattctgccctc

SEQ ID NO: 203 - DNA, 25 bp, synthetic construct
  source 1..25: mol_type = other DNA
gctccaatgcacccaagacagcaga

SEQ ID NO: 204 - DNA, 25 bp, synthetic construct
  source 1..25: mol_type = other DNA
agtagctgcgctgatagacatccat

SEQ ID NO: 205 - DNA, 25 bp, synthetic construct
  source 1..25: mol_type = other DNA
catggtgatgttggactcctcagtg

SEQ ID NO: 206 - DNA, 25 bp, synthetic construct
  source 1..25: mol_type = other DNA
cttcgtgatgattctgccctcctcc

SEQ ID NO: 207 - DNA, 25 bp, synthetic construct
  source 1..25: mol_type = other DNA
atctgcatggtgatgttggactcct

SEQ ID NO: 208 - DNA, 25 bp, synthetic construct
  source 1..25: mol_type = other DNA
caggccctcgtcattgcagcagccc

SEQ ID NO: 209 - DNA, 25 bp, synthetic construct
  source 1..25: mol_type = other DNA
tctgcatggtgatgttggactcctc

SEQ ID NO: 210 - DNA, 25 bp, synthetic construct
  source 1..25: mol_type = other DNA
tgcatggtgatgttggactcctcag

SEQ ID NO: 211 - DNA, 25 bp, synthetic construct
  source 1..25: mol_type = other DNA
tagagcagcaaggcaaggctccaat

SEQ ID NO: 212 - DNA, 25 bp, synthetic construct
  source 1..25: mol_type = other DNA
atgcacccaagacagcagaaagttc

SEQ ID NO: 213 - DNA, 25 bp, synthetic construct
  source 1..25: mol_type = other DNA
ccgcatcgcatcaggggcacacagg

SEQ ID NO: 214 - DNA, 25 bp, synthetic construct
  source 1..25: mol_type = other DNA
gctggccttggtgaggtttgatccg

SEQ ID NO: 215 - DNA, 25 bp, synthetic construct
  source 1..25: mol_type = other DNA
gtgctggccttggtgaggtttgatc

SEQ ID NO: 216 - DNA, 25 bp, synthetic construct
  source 1..25: mol_type = other DNA
atgtgctggccttggtgaggtttga

SEQ ID NO: 217 - DNA, 25 bp, synthetic construct
  source 1..25: mol_type = other DNA
ctatgtgctggccttggtgaggttt

SEQ ID NO: 218 - DNA, 25 bp, synthetic construct
  source 1..25: mol_type = other DNA
tcctatgtgctggccttggtgaggt

SEQ ID NO: 219 - DNA, 25 bp, synthetic construct
  source 1..25: mol_type = other DNA
tctcctatgtgctggccttggtgag

SEQ ID NO: 220 - DNA, 25 bp, synthetic construct
  source 1..25: mol_type = other DNA
tctctcctatgtgctggccttggtg

SEQ ID NO: 221 - DNA, 25 bp, synthetic construct
  source 1..25: mol_type = other DNA
catctctcctatgtgctggccttgg

SEQ ID NO: 222 - DNA, 25 bp, synthetic construct
  source 1..25: mol_type = other DNA
tcatctctcctatgtgctggccttg

SEQ ID NO: 223 - DNA, 25 bp, synthetic construct
  source 1..25: mol_type = other DNA
ctcatctctcctatgtgctggcctt

SEQ ID NO: 224 - DNA, 25 bp, synthetic construct
  source 1..25: mol_type = other DNA
gctcatctctcctatgtgctggcct

SEQ ID NO: 225 - DNA, 25 bp, synthetic construct
  source 1..25: mol_type = other DNA
tgctggccttggtgaggtttgatcc

SEQ ID NO: 226 - DNA, 25 bp, synthetic construct
  source 1..25: mol_type = other DNA
tatgtgctggccttggtgaggtttg

SEQ ID NO: 227 - DNA, 26 bp, synthetic construct
  source 1..26: mol_type = other DNA
cagcctgggaccacttggcatggtgg

SEQ ID NO: 228 - DNA, 25 bp, synthetic construct
  source 1..25: mol_type = other DNA
gcagcctgggaccacttggcatggt

SEQ ID NO: 229 - DNA, 21 bp, synthetic construct
  source 1..21: mol_type = other DNA
tgggtgcagcctgggaccact

SEQ ID NO: 230 - DNA, 28 bp, synthetic construct
  source 1..28: mol_type = other DNA
agcctgggaccacttggcatggtggagg

SEQ ID NO: 231 - DNA, 20 bp, synthetic construct
  source 1..20: mol_type = other DNA
tccaaaatcaagtggggcga

SEQ ID NO: 232 - DNA, 20 bp, synthetic construct
  source 1..20: mol_type = other DNA
tgatgacccttttggctccc

SEQ ID NO: 233 - DNA, 21 bp, synthetic construct
  source 1..21: mol_type = other DNA
tgtcacgtcctgcacgacgta

SEQ ID NO: 234 - DNA, 21 bp, synthetic construct
  source 1..21: mol_type = other DNA
ttcagcaccgcggacagtgcc

SEQ ID NO: 235 - DNA, 42 bp, synthetic construct
  source 1..42: mol_type = other DNA
ttcagcaccgcggacagtgcctgtcacgtcctgcacgacgta

SEQ ID NO: 236 - DNA, 96 bp, synthetic construct
  source 1..96: mol_type = other DNA
gtgctgtaggaagctcatctctcctatgtggctggagcagcccccgatttgtggggtgattacagcggtactcctggaagatgtccaccagggtct

SEQ ID NO: 237 - DNA, 25 bp, synthetic construct
  source 1..25: mol_type = other DNA
gaatgtagccatccatccttgtcaa

SEQ ID NO: 238 - DNA, 50 bp, synthetic construct
  source 1..50: mol_type = other DNA
tatgcggatcaaacctcaccaaggccagcacataggagagatgagcttcc

SEQ ID NO: 239 - DNA, 50 bp, synthetic construct
  source 1..50: mol_type = other DNA
ggaagctcatctctcctatgtgctggccttggtgaggtttgatccgcata

SEQ ID NO: 240 - DNA, 60 bp, synthetic construct
  source 1..60: mol_type = other DNA
gcccatgccttgctctctttctgtcctcagtggtcccaggctgcacccatggcagaagga

SEQ ID NO: 241 - DNA, 60 bp, synthetic construct
  source 1..60: mol_type = other DNA
tccttctgccatgggtgcagcctgggaccactgaggacagaaagagagcaaggcatgggc

SEQ ID NO: 242 - DNA, 65 bp, synthetic construct
  source 1..65: mol_type = other DNA
ttgccttgctgctctacctccaccatgccaagtggtcccaggctgcacccatggcagaaggagga

SEQ ID NO: 243 - DNA, 65 bp, synthetic construct
  source 1..65: mol_type = other DNA
tcctccttctgccatgggtgcagcctgggaccacttggcatggtggaggtagagcagcaaggcaa